European Patent Application EP 4 792 829 A1, published August 19, 2026. Title: Virus-based expression of proteins and genes. Applicant: Sagitta Biotech. Application EP. The sequence listing filed with the application follows.

SEQUENCE LISTING (21 sequences)

SEQ ID NO: 1 - DNA, 1524 bp, synthetic construct
  source 1..1524: mol_type = other DNA; note = P
  CDS 1..1524: protein_id = 2; translation = MAEEQARHVKNGLECIRALKAEPIGSLAIEEAMAAWSEISDNPGQERATCREEKAGSSGLSKPCLSAIGSTEGGAPRIRGQGPGESDDDAETLGIPPRNLQASSTGLQCYYVYDHSGEAVKGIQDADSIMVQSGLDGDSTLSGGDNESENSDVDIGEPDTEGYAITDRGSAPISMGFRASDVETAEGGEIHELLRLQSRGNNFPKLGKTLNVPPPPDPGRASTSGTPIKKGTDARLASFGTEIASLLTGGATQCARKSPSEPSGPGAPAGNVPECVSNAALIQEWTPESGTTISPRSQNNEEGGDYYDDELFSDVQDIKTALAKIHEDNQKIISKLESLLLLKGEVESIKKQINRQNISISTLEGHLSSIMIAIPGLGKDPNDPTADVEINPDLKPIIGRDSGRALAEVLKKPVASRQLQGMTNGRTSSRGQLLKEFQLKPIGKKMSSAVGFVPDTGPASRSVIRSIIKSSRLEEDRKRYLMTLLDDIKGANDLAKFHQMLMKIIMK
atggcagaagagcaggcacgccatgtcaaaaacggactggaatgcatccgggctctcaaggccgagcccatcggctcactggccatcgaggaagctatggcagcatggtcagaaatatcagacaacccaggacaggagcgagccacctgcagggaagagaaggcaggcagttcgggtctcagcaaaccatgcctctcagcaattggatcaactgaaggcggtgcacctcgcatccgcggtcagggacctggagagagcgatgacgacgctgaaactttgggaatccccccaagaaatctccaggcatcaagcactgggttacagtgttattatgtttatgatcacagcggtgaagcggttaagggaatccaagatgctgactctatcatggttcaatcaggccttgatggtgatagcaccctctcaggaggagacaatgaatctgaaaacagcgatgtggatattggcgaacctgataccgagggatatgctatcactgaccggggatctgctcccatctctatggggttcagggcttctgatgttgaaactgcagaaggaggggagatccacgagctcctgagactccaatccagaggcaacaactttccgaagcttgggaaaactctcaatgttcctccgcctccggaccccggtagggccagcacttccgggacacccattaaaaagggcacagacgcgagattagcctcatttggaacggagatcgcgtctttattgacaggtggtgcaacccaatgtgctcgaaagtcaccctcggaaccatcagggccaggtgcacctgcggggaatgtccccgagtgtgtgagcaatgccgcactgatacaggagtggacacccgaatctggtaccacaatctccccgagatcccagaataatgaagaagggggagactattatgatgatgagctgttctctgatgtccaagatattaaaacagccttggccaaaatacacgaggataatcagaagataatctccaagctagaatcactgctgttattgaagggagaagttgagtcaattaagaagcagatcaacaggcaaaatatcagcatatccaccctggaaggacacctctcaagcatcatgatcgccattcctggacttgggaaggatcccaacgaccccactgcagatgtcgaaatcaatcccgacttgaaacccatcataggcagagattcaggccgagcactggccgaagttctcaagaaacccgttgccagccgacaactccaaggaatgacaaatggacggaccagttccagaggacagctgctgaaggaatttcagctaaagccgatcgggaaaaagatgagctcagccgtcgggtttgttcctgacaccggccctgcatcacgcagtgtaatccgctccattataaaatccagccggctagaggaggatcggaagcgttacctgatgactctccttgatgatatcaaaggagccaatgatcttgccaagttccaccagatgctgatgaagataataatgaagtag

SEQ ID NO: 2 - protein, 507 aa, synthetic construct
MAEEQARHVKNGLECIRALKAEPIGSLAIEEAMAAWSEISDNPGQERATCREEKAGSSGLSKPCLSAIGSTEGGAPRIRGQGPGESDDDAETLGIPPRNLQASSTGLQCYYVYDHSGEAVKGIQDADSIMVQSGLDGDSTLSGGDNESENSDVDIGEPDTEGYAITDRGSAPISMGFRASDVETAEGGEIHELLRLQSRGNNFPKLGKTLNVPPPPDPGRASTSGTPIKKGTDARLASFGTEIASLLTGGATQCARKSPSEPSGPGAPAGNVPECVSNAALIQEWTPESGTTISPRSQNNEEGGDYYDDELFSDVQDIKTALAKIHEDNQKIISKLESLLLLKGEVESIKKQINRQNISISTLEGHLSSIMIAIPGLGKDPNDPTADVEINPDLKPIIGRDSGRALAEVLKKPVASRQLQGMTNGRTSSRGQLLKEFQLKPIGKKMSSAVGFVPDTGPASRSVIRSIIKSSRLEEDRKRYLMTLLDDIKGANDLAKFHQMLMKIIMK

SEQ ID NO: 3 - DNA, 1578 bp, synthetic construct
  source 1..1578: mol_type = other DNA; note = N
  CDS 1..1578: protein_id = 4; translation = MATLLRSLALFKRNKDKPPITSGSGGAIRGIKHIIIVPIPGDSSITTRSRLLDRLVRLIGNPDVSGPKLTGALIGILSLFVESPGQLIQRITDDPDVSIRLLEVVQSDQSQSGLTFASRGTNMEDEADQYFSHDDPISSDQSRFGWFENKEISDIEVQDPEGFNMILGTILAQIWVLLAKAVTAPDTAADSELRRWIKYTQQRRVVGEFRLERKWLDVVRNRIAEDLSLRRFMVALILDIKRTPGNKPRIAEMICDIDTYIVEAGLASFILTIKFGIETMYPALGLHEFAGELSTLESLMNLYQQMGETAPYMVILENSIQNKFSAGSYPLLWSYAMGVGVELENSMGGLNFGRSYFDPAYFRLGQEMVRRSAGKVSSTLASELGITAEDARLVSEIAMHTTEDKISRAVGPRQAQVSFLHGDQSENELPRLGGKEDRRVKQSRGEARESYRETGPSRASDARAAHLPTGTPLDIDTASESSQDPQDSRRSADALLRLQAMAGISEEQGSDTDTPIVYNDRNLLDG
atggccacacttttaaggagcttagcattgttcaaaagaaacaaggacaaaccacccattacatcaggatccggtggagccatcagaggaatcaaacacattattatagtaccaatccctggagattcctcaattaccactcgatccagacttctggaccggttggtcaggttaattggaaacccggatgtgagcgggcccaaactaacaggggcactaataggtatattatccttatttgtggagtctccaggtcaattgattcagaggatcaccgatgaccctgacgttagcataaggctgttagaggttgtccagagtgaccagtcacaatctggccttaccttcgcatcaagaggtaccaacatggaggatgaggcggaccaatacttttcacatgatgatccaattagtagtgatcaatccaggttcggatggttcgagaacaaggaaatctcagatattgaagtgcaagaccctgagggattcaacatgattctgggtaccatcctagctcaaatttgggtcttgctcgcaaaggcggttacggccccagacacggcagctgattcggagctaagaaggtggataaagtacacccaacaaagaagggtagttggtgaatttagattggagagaaaatggttggatgtggtgaggaacaggattgccgaggacctctccttacgccgattcatggtcgctctaatcctggatatcaagagaacacccggaaacaaacccaggattgctgaaatgatatgtgacattgatacatatatcgtagaggcaggattagccagttttatcctgactattaagtttgggatagaaactatgtatcctgctcttggactgcatgaatttgctggtgagttatccacacttgagtccttgatgaacctttaccagcaaatgggggaaactgcaccctacatggtaatcctggagaactcaattcagaacaagttcagtgcaggatcataccctctgctctggagctatgccatgggagtaggagtggaacttgaaaactccatgggaggtttgaactttggccgatcttactttgatccagcatattttagattagggcaagagatggtaaggaggtcagctggaaaggtcagttccacattggcatctgaactcggtatcactgccgaggatgcaaggcttgtttcagagattgcaatgcatactactgaggacaagatcagtagagcggttggacccagacaagcccaagtatcatttctacacggtgatcaaagtgagaatgagctaccgagattggggggcaaggaagataggagggtcaaacagagtcgaggagaagccagggagagctacagagaaaccgggcccagcagagcaagtgatgcgagagctgcccatcttccaaccggcacacccctagacattgacactgcatcggagtccagccaagatccgcaggacagtcgaaggtcagctgacgccctgcttaggctgcaagccatggcaggaatctcggaagaacaaggctcagacacggacacccctatagtgtacaatgacagaaatcttctagacggc

SEQ ID NO: 4 - protein, 526 aa, synthetic construct
MATLLRSLALFKRNKDKPPITSGSGGAIRGIKHIIIVPIPGDSSITTRSRLLDRLVRLIGNPDVSGPKLTGALIGILSLFVESPGQLIQRITDDPDVSIRLLEVVQSDQSQSGLTFASRGTNMEDEADQYFSHDDPISSDQSRFGWFENKEISDIEVQDPEGFNMILGTILAQIWVLLAKAVTAPDTAADSELRRWIKYTQQRRVVGEFRLERKWLDVVRNRIAEDLSLRRFMVALILDIKRTPGNKPRIAEMICDIDTYIVEAGLASFILTIKFGIETMYPALGLHEFAGELSTLESLMNLYQQMGETAPYMVILENSIQNKFSAGSYPLLWSYAMGVGVELENSMGGLNFGRSYFDPAYFRLGQEMVRRSAGKVSSTLASELGITAEDARLVSEIAMHTTEDKISRAVGPRQAQVSFLHGDQSENELPRLGGKEDRRVKQSRGEARESYRETGPSRASDARAAHLPTGTPLDIDTASESSQDPQDSRRSADALLRLQAMAGISEEQGSDTDTPIVYNDRNLLDG

SEQ ID NO: 5 - DNA, 6552 bp, synthetic construct
  source 1..6552: mol_type = other DNA
  CDS 1..6552: note = L; protein_id = 6; translation = MDSLSVNQILYPEVHLDSPIVTNKIVAILEYARVPHAYSLEDPTLCQNIKHRLKNGFSNQMIINNVEVGNVIKSKLRSYPAHSHIPYPNCNQDLFNIEDKESTRKIRELLKKGNSLYSKVSDKVFQCLRDTNSRLGLGSELREDIKEKVINLGVYMHSSQWFEPFLFWFTVKTEMRSVIKSQTHTCHRRRHTPVFFTGSSVELLISRDLVAIISKESQHVYYLTFELVLMYCDVIEGRLMTETAMTIDARYTELLGRVRYMWKLIDGFFPALGNPTYQIVAMLEPLSLAYLQLRDITVELRGAFLNHCFTEIHDVLDQNGFSDEGTYHELIEALDYIFITDDIHLTGEIFSFFRSFGHPRLEAVTAAENVRKYMNQPKVIVYETLMKGHAIFCGIIINGYRDRHGGSWPPLTLPLHAADTIRNAQASGEGLTHEQCVDNWRSFAGVKFGCFMPLSLDSDLTMYLKDKALAALQREWDSVYPKEFLRYDPPKGTGSRRLVDVFLNDSSFDPYDVIMYVVSGAYLHDPEFNLSYSLKEKEIKETGRLFAKMTYKMRACQVIAENLISNGIGKYFKDNGMAKDEHDLTKALHTLAVSGVPKDLKESHRGGPVLKTYSRSPVHTSTRNVRAAKGFIGFPQVIRQDQDTDHPENMEAYETVSAFITTDLKKYCLNWRYETISLFAQRLNEIYGLPSFFQWLHKRLETSVLYVSDPHCPPDLDAHIPLYKVPNDQIFIKYPMGGIEGYCQKLWTISTIPYLYLAAYESGVRIASLVQGDNQTIAVTKRVPSTWPYNLKKREAARVTRDYFVILRQRLHDIGHHLKANETIVSSHFFVYSKGIYYDGLLVSQSLKSIARCVFWSETIVDETRAACSNIATTMAKSIERGYDRYLAYSLNVLKVIQQILISLGFTINSTMTRDVVIPLLTNNDLLIRMALLPAPIGGMNYLNMSRLFVRNIGDPVTSSIADLKRMILASLMPEETLHQVMTQQPGDSSFLDWASDPYSANLVCVQSITRLLKNITARFVLIHSPNPMLKGLFHDDSKEEDEGLAAFLMDRHIIVPRAAHEILDHSVTGARESIAGMLDTTKGLIRASMRKGGLTSRVITRLSNYDYEQFRAGMVLLTGRKRNVLIDKESCSVQLARALRSHMWARLARGRPIYGLEVPDVLESMRGHLIRRHETCVICECGSVNYGWFFVPSGCQLDDIDKETSSLRVPYIGSTTDERTDMKLAFVRAPSRSLRSAVRIATVYSWAYGDDDSSWNEAWLLARQRANVSLEELRVITPISTSTNLAHRLRDRSTQVKYSGTSLVRVARYTTISNDNLSFVISDKKVDTNFIYQQGMLLGLGVLETLFRLEKDTGSSNTVLHLHVETDCCVIPMIDHPRIPSSRKLELRAELCTNPLIYDNAPLIDRDTTRLYTQSHRRHLVEFVTWSTPQLYHILAKSTALSMIDLVTKFEKDHMNEISALIGDDDINSFITEFLLIEPRLFTIYLGQCAAINWAFDVHYHRPSGKYQMGELLSSFLSRMSKGVFKVLVNALSHPKIYKKFWHCGIIEPIHGPSLDAQNLHTTVCNMVYTCYMTYLDLLLNEELEEFTFLLCESDEDVVPDRFDNIQAKHLCVLADLYCQPGTCPPIRGLRPVEKCAVLTDHIKAEARLSPAGSSWNINPIIVDHYSCSLTYLRRGSIKQIRLRVDPGFIFDALAEVNVSQPKIGSNNISNMSIKAFRPPHDDVAKLLKDINTSKHNLPISGGNLANYEIHAFRRIGLNSSACYKAVEISTLIRRCLEPGEDGLFLGEGSGSMLITYKEILKLNKCFYNSGVSANSRSGQRELAPYPSEVGLVEHRMGVGNIVKVLFNGRPEVTWVGSVDCFNFIVSNIPTSSVGFIHSDIETLPNKDTIEKLEELAAILSMALLLGKIGSILVIKLMPFSGDFVQGFISYVGSHYREVNLVYPRYSNFISTESYLVMTDLKANRLMNPEKIKQQIIESSVRTSPGLIGHILSIKQLSCIQAIVGDAVSRGDINPTLKKLTPIEQVLINCGLAINGPKLCKELIHHDVASGQDGLLNSILILYRELARFKDNQRSQQGMFHAYPVLVSSRQRELISRITRKFWGHILLYSGNRKLINKFIQNLKSGYLILDLHQNIFVKNLSKSEKQIIMTGGLKREWVFKVTVKETKEWYKLVGYSALIKD
atggactcgctatctgtcaaccagatcttataccctgaagttcacctagatagcccgatagttaccaataagatagtagccatcctggagtatgctcgagtccctcacgcttacagcctggaggaccctacactgtgtcagaacatcaagcaccgcctaaaaaacggattttccaaccaaatgattataaacaatgtggaagttgggaatgtcatcaagtccaagcttaggagttatccggcccactctcatattccatatccaaattgtaatcaggatttatttaacatagaagacaaagagtcaacgaggaagatccgtgaactcctcaaaaaggggaattcgctgtactccaaagtcagtgataaggttttccaatgcttaagggacactaactcacggcttggcctaggctccgaattgagggaggacatcaaggagaaagttattaacttgggagtttacatgcacagctcccagtggtttgagccctttctgttttggtttacagtcaagactgagatgaggtcagtgattaaatcacaaacccatacttgccataggaggagacacacacctgtattcttcactggtagttcagttgagttgctaatctctcgtgaccttgttgctataatcagtaaagagtctcaacatgtatattacctgacatttgaactggttttgatgtattgtgatgtcatagaggggaggttaatgacagagaccgctatgactattgatgctaggtatacagagcttctaggaagagtcagatacatgtggaaactgatagatggtttcttccctgcactcgggaatccaacttatcaaattgtagccatgctggagcctctttcacttgcttacctgcagctgagggatataacagtagaactcagaggtgctttccttaaccactgctttactgaaatacatgatgttcttgaccaaaacgggttttctgatgaaggtacttatcatgagttaattgaagctctagattacattttcataactgatgacatacatctgacaggggagattttctcatttttcagaagtttcggccaccccagacttgaagcagtaacggctgctgaaaatgttaggaaatacatgaatcagcctaaagtcattgtgtatgagactctgatgaaaggtcatgccatattttgtggaatcataatcaacggctatcgtgacaggcacggaggcagttggccaccgctgaccctccccctgcatgctgcagacacaatccggaatgctcaagcttcaggtgaagggttaacacatgagcagtgcgttgataactggagatcttttgctggagtgaaatttggctgctttatgcctcttagcctggatagtgatctgacaatgtacctaaaggacaaggcacttgctgctctccaaagggaatgggattcagtttacccgaaagagttcctgcgttacgaccctcccaagggaaccgggtcacggaggcttgtagatgttttccttaatgattcgagctttgacccatatgatgtgataatgtatgttgtaagtggagcttacctccatgaccctgagttcaacctgtcttacagcctgaaagaaaaggagatcaaggaaacaggtagactttttgctaaaatgacttacaaaatgagggcatgccaagtgattgctgaaaatctaatctcaaacgggattggcaaatattttaaggacaatgggatggccaaggatgagcacgatttgactaaggcactccacactctagctgtctcaggagtccccaaagatctcaaagaaagtcacaggggggggccagtcttaaaaacctactcccgaagcccagtccacacaagtaccaggaacgtgagagcagcaaaagggtttatagggttccctcaagtaattcggcaggaccaagacactgatcatccggagaatatggaagcttacgagacagtcagtgcatttatcacgactgatctcaagaagtactgccttaattggagatatgagaccatcagcttgtttgcacagaggctaaatgagatttacggattgccctcatttttccagtggctgcataagaggcttgagacctctgtcctgtatgtaagtgaccctcattgcccccccgaccttgacgcccatatcccgttatataaagtccccaatgatcaaatcttcattaagtaccctatgggaggtatagaagggtattgtcagaagctgtggaccatcagcaccattccctatctatacctggctgcttatgagagcggagtaaggattgcttcgttagtgcaaggggacaatcagaccatagccgtaacaaaaagggtacccagcacatggccctacaaccttaagaaacgggaagctgctagagtaactagagattactttgtaattcttaggcaaaggctacatgatattggccatcacctcaaggcaaatgagacaattgtttcatcacatttttttgtctattcaaaaggaatatattatgatgggctacttgtgtcccaatcactcaagagcatcgcaagatgtgtattctggtcagagactatagttgatgaaacaagggcagcatgcagtaatattgctacaacaatggctaaaagcatcgagagaggttatgaccgttaccttgcatattccctgaacgtcctaaaagtgatacagcaaattctgatctctcttggcttcacaatcaattcaaccatgacccgggatgtagtcatacccctcctcacgaacaacgacctcttaataaggatggcactgttgcccgctcctattggggggatgaattatctgaatatgagcaggctgtttgtcagaaacatcggtgatccagtaacatcatcaattgctgatctcaagagaatgattctcgcctcactaatgcctgaagagaccctccatcaagtaatgacacaacaaccgggggactcttcattcctagactgggctagcgacccttactcagcaaatcttgtatgtgtccagagcatcactagactcctcaagaacataactgcaaggtttgtcctgatccatagtccaaacccaatgttaaaaggattattccatgatgacagtaaagaagaggacgagggactggcggcattcctcatggacaggcatattatagtacctagggcagctcatgaaatcctggatcatagtgtcacaggggcaagagagtctattgcaggcatgctggataccacaaaaggcctgattcgagccagcatgaggaagggggggttaacctctcgagtgataaccagattgtccaattatgactatgaacaattcagagcagggatggtgctattgacaggaagaaagagaaatgtcctcattgacaaagagtcatgttcagtgcagctggcgagagctctaagaagccatatgtgggcgaggctagctcgaggacggcctatttacggccttgaggtccctgatgtactagaatctatgcgaggccaccttattcggcgtcatgagacatgtgtcatctgcgagtgtggatcagtcaactacggatggttttttgtcccctcgggttgccaactggatgatattgacaaggaaacatcatccttgagagtcccatatattggttctaccactgatgagagaacagacatgaagcttgccttcgtaagagccccaagtcgatccttgcgatctgctgttagaatagcaacagtgtactcatgggcttacggtgatgatgatagctcttggaacgaagcctggttgttggctaggcaaagggccaatgtgagcctggaggagctaagggtgatcactcccatctcaacttcgactaatttagcgcataggttgagggatcgtagcactcaagtgaaatactcaggtacatcccttgtccgagtggcgaggtataccacaatctccaacgacaatctctcatttgtcatatcagataagaaggttgatactaactttatataccaacaaggaatgcttctagggttgggtgttttagaaacattgtttcgactcgagaaagataccggatcatctaacacggtattacatcttcacgtcgaaacagattgttgcgtgatcccgatgatagatcatcccaggatacccagctcccgcaagctagagctgagggcagagctatgtaccaacccattgatatatgataatgcacctttaattgacagagatacaacaaggctatacacccagagccataggaggcaccttgtggaatttgttacatggtccacaccccaactatatcacattttagctaagtccacagcactatctatgattgacctggtaacaaaatttgagaaggaccatatgaatgaaatttcagctctcataggggatgacgatatcaatagtttcataactgagtttctgctcatagagccaagattattcactatctacttgggccagtgtgcggccatcaattgggcatttgatgtacattatcatagaccatcagggaaatatcagatgggtgagctgttgtcatcgttcctttctagaatgagcaaaggagtgtttaaggtgcttgtcaatgctctaagccacccaaagatctacaagaaattctggcattgtggtattatagagcctatccatggtccttcacttgatgctcaaaacttgcacacaactgtgtgcaacatggtttacacatgctatatgacctacctcgacctgttgttgaatgaagagttagaagagttcacatttctcttgtgtgaaagcgacgaggatgtagtaccggacagattcgacaacatccaggcaaaacacttatgtgttctggcagatttgtactgtcaaccagggacctgcccaccaattcgaggtctaagaccggtagagaaatgtgcagttctaaccgaccatatcaaggcagaggctaggttatctccagcaggatcttcgtggaacataaatccaattattgtagaccattactcatgctctctgacttatctccggcgaggatcgatcaaacagataagattgagagttgatccaggattcattttcgacgccctcgctgaggtaaatgtcagtcagccaaagatcggcagcaacaacatctcaaatatgagcatcaaggctttcagacccccacacgatgatgttgcaaaattgctcaaagatatcaacacaagcaagcacaatcttcccatttcagggggcaatctcgccaattatgaaatccatgctttccgcagaatcgggttgaactcatctgcttgctacaaagctgttgagatatcaacattaattaggagatgccttgagccaggggaggacggcttgttcttgggtgagggatcgggttccatgttgatcacttataaggagatacttaaactaaacaagtgcttctataatagtggggtttccgccaattctagatctggtcaaagggaattagcaccctatccctccgaagttggccttgtcgaacacagaatgggagtaggtaatattgtcaaagtgctctttaacgggaggcccgaagtcacgtgggtaggcagtgtagattgcttcaatttcatagttagtaatatccctacctctagtgtggggtttatccattcagatatagagaccttgcctaacaaagatactatagagaagctagaggaattggcagccatcttatcgatggctctgctcctgggcaaaataggatcaatactggtgattaagcttatgcctttcagcggggattttgttcagggatttataagttatgtagggtcccattatagagaagtgaaccttgtataccctagatacagcaacttcatatctactgaatcttatttggttatgacagatctcaaggctaaccggctaatgaatcctgaaaagattaagcagcagataattgaatcatctgtgaggacttcacctggacttataggtcacatcctatccattaagcaactaagctgcatacaagcaattgtgggagacgcagttagtagaggtgatatcaatcctactctgaaaaaacttacacctatagagcaggtgctgatcaattgcgggttggcaattaacggacctaagctgtgcaaagaattgatccaccatgatgttgcctcagggcaagatggattgcttaattctatactcatcctctacagggagttggcaagattcaaagacaaccaaagaagtcaacaagggatgttccacgcttaccccgtattggtaagtagcaggcaacgagaacttatatctaggatcacccgcaaattttgggggcacattcttctttactccgggaacagaaagttgataaataagtttatccagaatctcaagtccggctatctgatactagacttacaccagaatatcttcgttaagaatctatccaagtcagagaaacagattattatgacggggggtttgaaacgtgagtgggtttttaaggtaacagtcaaggagaccaaagaatggtataagttagtcggatacagtgccctgattaaggactaa

SEQ ID NO: 6 - protein, 2183 aa, synthetic construct
MDSLSVNQILYPEVHLDSPIVTNKIVAILEYARVPHAYSLEDPTLCQNIKHRLKNGFSNQMIINNVEVGNVIKSKLRSYPAHSHIPYPNCNQDLFNIEDKESTRKIRELLKKGNSLYSKVSDKVFQCLRDTNSRLGLGSELREDIKEKVINLGVYMHSSQWFEPFLFWFTVKTEMRSVIKSQTHTCHRRRHTPVFFTGSSVELLISRDLVAIISKESQHVYYLTFELVLMYCDVIEGRLMTETAMTIDARYTELLGRVRYMWKLIDGFFPALGNPTYQIVAMLEPLSLAYLQLRDITVELRGAFLNHCFTEIHDVLDQNGFSDEGTYHELIEALDYIFITDDIHLTGEIFSFFRSFGHPRLEAVTAAENVRKYMNQPKVIVYETLMKGHAIFCGIIINGYRDRHGGSWPPLTLPLHAADTIRNAQASGEGLTHEQCVDNWRSFAGVKFGCFMPLSLDSDLTMYLKDKALAALQREWDSVYPKEFLRYDPPKGTGSRRLVDVFLNDSSFDPYDVIMYVVSGAYLHDPEFNLSYSLKEKEIKETGRLFAKMTYKMRACQVIAENLISNGIGKYFKDNGMAKDEHDLTKALHTLAVSGVPKDLKESHRGGPVLKTYSRSPVHTSTRNVRAAKGFIGFPQVIRQDQDTDHPENMEAYETVSAFITTDLKKYCLNWRYETISLFAQRLNEIYGLPSFFQWLHKRLETSVLYVSDPHCPPDLDAHIPLYKVPNDQIFIKYPMGGIEGYCQKLWTISTIPYLYLAAYESGVRIASLVQGDNQTIAVTKRVPSTWPYNLKKREAARVTRDYFVILRQRLHDIGHHLKANETIVSSHFFVYSKGIYYDGLLVSQSLKSIARCVFWSETIVDETRAACSNIATTMAKSIERGYDRYLAYSLNVLKVIQQILISLGFTINSTMTRDVVIPLLTNNDLLIRMALLPAPIGGMNYLNMSRLFVRNIGDPVTSSIADLKRMILASLMPEETLHQVMTQQPGDSSFLDWASDPYSANLVCVQSITRLLKNITARFVLIHSPNPMLKGLFHDDSKEEDEGLAAFLMDRHIIVPRAAHEILDHSVTGARESIAGMLDTTKGLIRASMRKGGLTSRVITRLSNYDYEQFRAGMVLLTGRKRNVLIDKESCSVQLARALRSHMWARLARGRPIYGLEVPDVLESMRGHLIRRHETCVICECGSVNYGWFFVPSGCQLDDIDKETSSLRVPYIGSTTDERTDMKLAFVRAPSRSLRSAVRIATVYSWAYGDDDSSWNEAWLLARQRANVSLEELRVITPISTSTNLAHRLRDRSTQVKYSGTSLVRVARYTTISNDNLSFVISDKKVDTNFIYQQGMLLGLGVLETLFRLEKDTGSSNTVLHLHVETDCCVIPMIDHPRIPSSRKLELRAELCTNPLIYDNAPLIDRDTTRLYTQSHRRHLVEFVTWSTPQLYHILAKSTALSMIDLVTKFEKDHMNEISALIGDDDINSFITEFLLIEPRLFTIYLGQCAAINWAFDVHYHRPSGKYQMGELLSSFLSRMSKGVFKVLVNALSHPKIYKKFWHCGIIEPIHGPSLDAQNLHTTVCNMVYTCYMTYLDLLLNEELEEFTFLLCESDEDVVPDRFDNIQAKHLCVLADLYCQPGTCPPIRGLRPVEKCAVLTDHIKAEARLSPAGSSWNINPIIVDHYSCSLTYLRRGSIKQIRLRVDPGFIFDALAEVNVSQPKIGSNNISNMSIKAFRPPHDDVAKLLKDINTSKHNLPISGGNLANYEIHAFRRIGLNSSACYKAVEISTLIRRCLEPGEDGLFLGEGSGSMLITYKEILKLNKCFYNSGVSANSRSGQRELAPYPSEVGLVEHRMGVGNIVKVLFNGRPEVTWVGSVDCFNFIVSNIPTSSVGFIHSDIETLPNKDTIEKLEELAAILSMALLLGKIGSILVIKLMPFSGDFVQGFISYVGSHYREVNLVYPRYSNFISTESYLVMTDLKANRLMNPEKIKQQIIESSVRTSPGLIGHILSIKQLSCIQAIVGDAVSRGDINPTLKKLTPIEQVLINCGLAINGPKLCKELIHHDVASGQDGLLNSILILYRELARFKDNQRSQQGMFHAYPVLVSSRQRELISRITRKFWGHILLYSGNRKLINKFIQNLKSGYLILDLHQNIFVKNLSKSEKQIIMTGGLKREWVFKVTVKETKEWYKLVGYSALIKD

SEQ ID NO: 7 - DNA, 57 bp, synthetic construct
  source 1..57: mol_type = other DNA; note = P2A
gccacgaacttctctctgttaaagcaagcaggagatgttgaagaaaaccccgggcct

SEQ ID NO: 8 - DNA, 121 bp, synthetic construct
  source 1..121: mol_type = other DNA; note = Intergene 1 MV
gtgcgagaggccgaggaccagaacaacatccgcctaccctccatcattgttataaaaaacttaggaaccaggtccacacagccgccagcccatcaaccatccactcccacgattggagccg

SEQ ID NO: 9 - DNA, 107 bp, synthetic construct
  source 1..107: mol_type = other DNA; note = Intergene 2 MV
ctacagctcaacttacctgccaaccccatgccagtcgacccaactagtacaacctaaatccattataaaaaacttaggagcaaagtgattgcctcccaagttccaca

SEQ ID NO: 10 - DNA, 109 bp, synthetic construct
  source 1..109: mol_type = other DNA; note = Intergene 5 MV
ggctgctagtgaaccaatctcatgatgtcacccagacatcaggcatacccactagtgtgaaatagacatcagaattaagaaaaacgtagggtccaagtggttccccgtt

SEQ ID NO: 11 - DNA, 109 bp, synthetic construct
  source 1..109: mol_type = other DNA; note = 5' NCT (5' Non coding region; end MV)
ttggttgaactccggaaccctaatcctgccctaggtggttaggcattatttgcaatagattaaagaaaactttgaaaatacgaagtttctattcccagctttgtctggt

SEQ ID NO: 12 - DNA, 1008 bp, synthetic construct
  source 1..1008: mol_type = other DNA
  CDS 1..1008: note = M (Matrix protein); protein_id = 13; translation = MTEIYDFDKSAWDIKGLIAPIQPTTYSDGRLVPQVRVIDPGLGDRKDECFMYMFLLGVVEDSDPLGPPIGRAFGSLPLGVGRSTAKPEKLLKEATELDIVVRRTAGLNEKLVFYNNTPLTLLTPWRKVLTTGSVFNANQVCNAVNLIPLDTPQRFRVVYMSITRLSDNGYYTVPRRMLEFRSVNAVAFNLLVTLRIDKAIGPGKIIDNTEQLPEATFMVHIGNFRRKKSEVYSADYCKMKIEKMGLVFALGGIGGTSLHIRSTGKMSKTLHAQLGFKKTLCYPLIDINEDLNRLLWRSRCKIVRIQAVLQPSVPQEFRIYDDVIINDDQGLFKVL
atgacagagatctacgacttcgacaagtcggcatgggacatcaaagggttgatcgctccgatacaacccaccacctacagtgatggcaggctggtgccccaggtcagagtcatagatcctggtctaggcgacaggaaggatgaatgctttatgtacatgtttctgctgggggttgttgaggacagcgatcccctagggcctccaatcgggcgagcatttgggtccctgcccttaggtgttggcagatccacagcaaagcccgaaaaactcctcaaagaggccactgagcttgacatagttgttagacgtacagcagggctcaatgaaaaactggtgttctacaacaacaccccactaactctcctcacaccttggagaaaggtcctaacaacagggagtgtcttcaacgcaaaccaagtgtgcaatgcggttaatctgataccgctcgataccccgcagaggttccgtgttgtttatatgagcatcacccgtctttcggataacgggtattacaccgttcctagaagaatgctggaattcagatcggtcaatgcagtggccttcaacctgctggtgacccttaggattgacaaggcgataggccctgggaagatcatcgacaatacagagcaacttcctgaggcaacatttatggtccacatcgggaacttcaggagaaagaagagtgaagtctactctgccgattattgcaaaatgaaaatcgaaaagatgggcctggtttttgcacttggtgggatagggggcaccagtcttcacattagaagcacaggcaaaatgagcaagactctccatgcacaactcgggttcaagaagaccttatgttacccgctgatagatatcaatgaagaccttaatcgattactctggaggagcagatgcaagatagtaagaatccaggcagttttgcagccatcagttcctcaagaattccgcatttacgacgacgtgatcataaatgatgaccaaggactattcaaagttctgtag

SEQ ID NO: 13 - protein, 335 aa, synthetic construct
MTEIYDFDKSAWDIKGLIAPIQPTTYSDGRLVPQVRVIDPGLGDRKDECFMYMFLLGVVEDSDPLGPPIGRAFGSLPLGVGRSTAKPEKLLKEATELDIVVRRTAGLNEKLVFYNNTPLTLLTPWRKVLTTGSVFNANQVCNAVNLIPLDTPQRFRVVYMSITRLSDNGYYTVPRRMLEFRSVNAVAFNLLVTLRIDKAIGPGKIIDNTEQLPEATFMVHIGNFRRKKSEVYSADYCKMKIEKMGLVFALGGIGGTSLHIRSTGKMSKTLHAQLGFKKTLCYPLIDINEDLNRLLWRSRCKIVRIQAVLQPSVPQEFRIYDDVIINDDQGLFKVL

SEQ ID NO: 14 - DNA, 107 bp, synthetic construct
  source 1..107: mol_type = other DNA; note = 3' NCT (3' Non coding terminal region)
accaaacaaagttgggtaaggatagttcaatcaatgatcattttctagtgcacttaggattcaagatcctattatcagggacaagagcaggattaaggatatccgag

SEQ ID NO: 15 - DNA, 41 bp, synthetic construct
  source 1..41: mol_type = other DNA; note = Hammerhead ribozyme
ctgatgagtccgtgaggacgaaacggagtctagactccgtc

SEQ ID NO: 16 - DNA, 89 bp, synthetic construct
  source 1..89: mol_type = other DNA; note = Hepatitis C delta ribozyme
gggtcggcatggcatctccacctcctcgcggtccgacctgggcatccgaaggaggacgtacgtccactcggatggctaagggagagcca

SEQ ID NO: 17 - DNA, 19 bp, synthetic construct
  source 1..19: mol_type = other DNA; note = T7
taatacgactcactatagg

SEQ ID NO: 18 - DNA, 160 bp, synthetic construct
  source 1..160: mol_type = other DNA; note = MV Intergene 4
tcctctacaactcttgaaacacaaatgtcccacaagtctcctcttcgtcatcaagcaaccaccgcacccagcatcaagcccacctgaaattatctccggcttccctctggccgaacaatatcggtagttaattaaaacttagggtgcaagatcatccaca

SEQ ID NO: 19 - DNA, 134 bp, unidentified
  source 1..134: mol_type = genomic DNA; note = MV Intergene 3
ctacagctcaacttacctgccaaccccatgccagtcgacccaactagtacaacctaaatccattataaaaaacttaggaaccaggtccacacagccgccagcccatcaaccatccactcccacgattggagccg

SEQ ID NO: 20 - DNA, 54 bp, synthetic construct
  source 1..54: mol_type = other DNA; note = T2A
gagggcagaggaagtctgctaacatgcggtgacgtcgaggagaatcctggacct

SEQ ID NO: 21 - DNA, 37 bp, synthetic construct
  source 1..37: mol_type = other DNA; note = Varient HH
ctgatgaggccgaaaggccgaaactccgtaaggagtc